European Patent Application EP 4 512 414 A1, published February 26, 2025. Title: A combination therapy of GLP-2, and an insulinotropic peptide, TNFα inhibitor, or both for preventing or treating intestinal diseas. Applicant: HANMI PHARM. CO., LTD. The sequence listing filed with the application follows.

SEQUENCE LISTING (37 sequences)

SEQ ID NO: 1 - protein, 33 aa, Homo sapiens
HADGSFSDEMNTILDNLAARDFINWLIQTKITD

SEQ ID NO: 2 - protein, 34 aa, synthetic construct
  REGION 1..34: note = GLP-2 derivative
  SITE 1: note = MISC_FEATURE - Xaa is imidazoacetyldeshistidine
XGDGSFSDEMNTILDNLAARDFINWLIQTKITDC

SEQ ID NO: 3 - protein, 34 aa, synthetic construct
  REGION 1..34: note = GLP-2 derivative
  SITE 1: note = MISC_FEATURE - Xaa is imidazoacetyldeshistidine
XGDGSFSDEMNTILDNLAARDFINWLIQTKITDK

SEQ ID NO: 4 - protein, 34 aa, synthetic construct
  REGION 1..34: note = GLP-2 derivative
  SITE 1: note = MISC_FEATURE - Xaa is imidazoacetyldeshistidine
XGDGSFSDEMNTILDNLAARDFINWLIQTRITDK

SEQ ID NO: 5 - protein, 34 aa, synthetic construct
  REGION 1..34: note = GLP-2 derivative
  SITE 1: note = MISC_FEATURE - Xaa is imidazoacetyldeshistidine
  SITE 34: note = MISC_FEATURE - Xaa is 6-azidolysine
XGDGSFSDEMNTILDNLAARDFINWLIQTKITDX

SEQ ID NO: 6 - protein, 34 aa, synthetic construct
  REGION 1..34: note = GLP-2 derivative
  SITE 1: note = MISC_FEATURE - Xaa is imidazoacetyldeshistidine
XGDGSFSDEMNTILDNLAARDFINWLIQTRITDC

SEQ ID NO: 7 - protein, 34 aa, synthetic construct
  REGION 1..34: note = GLP-2 derivative
  SITE 1: note = MISC_FEATURE - Xaa is imidazoacetyldeshistidine
  SITE 2: note = MISC_FEATURE - Xaa is Aib(2-aminoisobutyric acid)
XXDGSFSDEMNTILDNLAARDFINWLIQTKITDC

SEQ ID NO: 8 - protein, 34 aa, synthetic construct
  REGION 1..34: note = GLP-2 derivative
  SITE 2: note = MISC_FEATURE - Xaa is Aib(2-aminoisobutyric acid)
HXDGSFSDEMNTILDNLAARDFINWLIQTKITDC

SEQ ID NO: 9 - protein, 34 aa, synthetic construct
  REGION 1..34: note = GLP-2 derivative
  SITE 1: note = MISC_FEATURE - Xaa = Histidine, imidazoacetyldeshistidine, desaminohistidine, beta-hydroxyimidazopropionyldeshistidine, N-dimethylhistidine, or beta-carboxyimidazopropionyldeshistidine
  SITE 2: note = MISC_FEATURE - Xaa is Alanine, Glycine, or Aib(2-aminoisobutyric acid)
  SITE 30: note = MISC_FEATURE - Xaa is Lysine, or Arginine
  SITE 34: note = MISC_FEATURE - Xaa is absent, Lysine, Arginine, Glutamine, Histidine, 6-azidolysine, or Cysteine
XXDGSFSDEMNTILDNLAARDFINWLIQTXITDX

SEQ ID NO: 10 - protein, 34 aa, synthetic construct; identical to SEQ ID NO: 9
  REGION 1..34: note = GLP-2 derivative
  SITE 1: note = MISC_FEATURE - Xaa = Histidine, imidazoacetyldeshistidine, desaminohistidine, beta-hydroxyimidazopropionyldeshistidine, N-dimethylhistidine, or beta-carboxyimidazopropionyldeshistidine
  SITE 2: note = MISC_FEATURE - Xaa is Alanine, Glycine, or Aib(2-aminoisobutyric acid)
  SITE 30: note = MISC_FEATURE - Xaa is Lysine, or Arginine
  SITE 34: note = MISC_FEATURE - Xaa = any one or more amino acid or any one or more amino acid which is modified

SEQ ID NO: 11 - protein, 12 aa, HOMO SAPIENS
ESKYGPPCPSCP

SEQ ID NO: 12 - protein, 11 aa, synthetic construct
  REGION 1..11: note = Variant of hinge region
ESKYGPPPSCP

SEQ ID NO: 13 - protein, 11 aa, synthetic construct
  REGION 1..11: note = Variant of hinge region
ESKYGPPCPSP

SEQ ID NO: 14 - protein, 10 aa, synthetic construct
  REGION 1..10: note = Variant of hinge region
ESKYGPPCPS

SEQ ID NO: 15 - protein, 10 aa, synthetic construct
  REGION 1..10: note = Variant of hinge region
ESKYGPPCPP

SEQ ID NO: 16 - protein, 8 aa, synthetic construct
  REGION 1..8: note = Variant of hinge region
KYGPPCPS

SEQ ID NO: 17 - protein, 8 aa, synthetic construct
  REGION 1..8: note = Variant of hinge region
ESKYGPPC

SEQ ID NO: 18 - protein, 7 aa, synthetic construct
  REGION 1..7: note = Variant of hinge region
EKYGPPC

SEQ ID NO: 19 - protein, 6 aa, synthetic construct
  REGION 1..6: note = Variant of hinge region
ESPSCP

SEQ ID NO: 20 - protein, 5 aa, synthetic construct
  REGION 1..5: note = Variant of hinge region
EPSCP

SEQ ID NO: 21 - protein, 4 aa, synthetic construct
  REGION 1..4: note = Variant of hinge region
PSCP

SEQ ID NO: 22 - protein, 10 aa, synthetic construct
  REGION 1..10: note = Variant of hinge region
ESKYGPPSCP

SEQ ID NO: 23 - protein, 9 aa, synthetic construct
  REGION 1..9: note = Variant of hinge region
KYGPPPSCP

SEQ ID NO: 24 - protein, 9 aa, synthetic construct
  REGION 1..9: note = Variant of hinge region
ESKYGPSCP

SEQ ID NO: 25 - protein, 8 aa, synthetic construct
  REGION 1..8: note = Variant of hinge region
ESKYGPPC

SEQ ID NO: 26 - protein, 7 aa, synthetic construct
  REGION 1..7: note = Variant of hinge region
KYGPPCP

SEQ ID NO: 27 - protein, 7 aa, synthetic construct
  REGION 1..7: note = Variant of hinge region
ESKPSCP

SEQ ID NO: 28 - protein, 6 aa, synthetic construct
  REGION 1..6: note = Variant of hinge region
ESPSCP

SEQ ID NO: 29 - protein, 4 aa, synthetic construct
  REGION 1..4: note = Variant of hinge region
EPSC

SEQ ID NO: 30 - skipped

SEQ ID NO: 31 - protein, 221 aa, homo sapiens
PSCPAPEFLGGPSVFLFPPKPKDTLMISRTPEVTCVVVDVSQEDPEVQFNWYVDGVEVHNAKTKPREEQFNSTYRVVSVLTVLHQDWLNGKEYKCKVSNKGLPSSIEKTISKAKGQPREPQVYTLPPSQEEMTKNQVSLTCLVKGFYPSDIAVEWESNGQPENNYKTTPPVLDSDGSFFLYSRLTVDKSRWQEGNVFSCSVMHEALHNHYTQKSLSLSLGK

SEQ ID NO: 32 - protein, 31 aa, synthetic construct
  REGION 1..31: note = GLP-1(7-37)
HAEGTFTSDVSSYLEGQAAKEFIAWLVKGRG

SEQ ID NO: 33 - protein, 39 aa, synthetic construct
  REGION 1..39: note = Exendin-3
HSDGTFTSDLSKQMEEEAVRLFIEWLKNGGPSSGAPPPS

SEQ ID NO: 34 - protein, 39 aa, synthetic construct
  REGION 1..39: note = Exendin-4
HGEGTFTSDLSKQMEEEAVRLFIEWLKNGGPSSGAPPPS

SEQ ID NO: 35 - protein, 442 aa, Homo sapiens
  REGION 1..442: note = MISC_FEATURE - Amino acids at position 1 to 442 form Human Immunoglobulin G4 Fc Fragment (homodimer)
  REGION 1..221: note = MISC_FEATURE - Amino acids at position 1 to 221 form one monomer
  REGION 222..442: note = MISC_FEATURE - Amino acids at position 222 to 442 form one monomer
  DISULFID 3..224: note = Amino acids at position 3 and position 224 form an inter-disulfide bond
  DISULFID 35..95: note = Amino acids at position 35 and position 95 form an intra-chain disulfide bond
  DISULFID 141..199: note = Amino acids at position 141 and position 199 form an intra-chain disulfide bond
  DISULFID 256..316: note = Amino acids at position 256 and position 316 form an intra-chain disulfide bond
  DISULFID 362..420: note = Amino acids at position 362 and position 420 form an intra-chain disulfide bond
PSCPAPEFLGGPSVFLFPPKPKDTLMISRTPEVTCVVVDVSQEDPEVQFNWYVDGVEVHNAKTKPREEQFNSTYRVVSVLTVLHQDWLNGKEYKCKVSNKGLPSSIEKTISKAKGQPREPQVYTLPPSQEEMTKNQVSLTCLVKGFYPSDIAVEWESNGQPENNYKTTPPVLDSDGSFFLYSRLTVDKSRWQEGNVFSCSVMHEALHNHYTQKSLSLSLGKPSCPAPEFLGGPSVFLFPPKPKDTLMISRTPEVTCVVVDVSQEDPEVQFNWYVDGVEVHNAKTKPREEQFNSTYRVVSVLTVLHQDWLNGKEYKCKVSNKGLPSSIEKTISKAKGQPREPQVYTLPPSQEEMTKNQVSLTCLVKGFYPSDIAVEWESNGQPENNYKTTPPVLDSDGSFFLYSRLTVDKSRWQEGNVFSCSVMHEALHNHYTQKSLSLSLGK

SEQ ID NO: 36 - protein, 4 aa, synthetic construct
  REGION 1..4: note = Linker
GGGS

SEQ ID NO: 37 - protein, 5 aa, synthetic construct
  REGION 1..5: note = Linker
GGGGS